European Patent Application EP 4 119 581 A1, published January 18, 2023. Title: Novel Fab dimers. Applicant: Helmholtz Zentrum Muenchen. The sequence listing filed with the application follows.

SEQUENCE LISTING (21 sequences)

SEQ ID NO: 1 - protein, 10 aa, artificial
  VH-CDR1
GFSLTTYSVS

SEQ ID NO: 2 - protein, 9 aa, artificial
  VH-CDR2
RMWYDGDTV

SEQ ID NO: 3 - protein, 13 aa, artificial
  VH-CDR3
DFGYFDGSSPFDY

SEQ ID NO: 4 - protein, 11 aa, artificial
  VL-CDR1
RASQGISTSIH

SEQ ID NO: 5 - protein, 7 aa, artificial
  VL-CDR2
FASQSIS

SEQ ID NO: 6 - protein, 10 aa, artificial
  VL-CDR3
QQTYSLPYTF

SEQ ID NO: 7 - protein, 229 aa, artificial
  VH of Fab6A10
QVQLKESGPGLVQPSETLSLTCTVSGFSLTTYSVSWVRQPSGKGPEWMGRMWYDGDTVYNSALKSRLSISRDTSKNQVFLKMNSLETDETGTYYCTRDFGYFDGSSPFDYWGQGVMVTVSSASTKGPSVFPLAPSSKSTSGGTAALGCLVKDYFPEPVTVSWNSGALTSGVHTFPAVLQSSGLYSLSSVVTVPSSSLGTQTYICNVNHKPSNTKVDKKVEPKSCDKTHT

SEQ ID NO: 8 - protein, 218 aa, artificial
  VL of Fab6A10
RCPVDIVLTQSPATLSVTPGESVSLSCRASQGISTSIHWYQQKSNESPRLLIKFASQSISGIPSRFSGSGSGTDFTLSINRVESEDFSVYFCQQTYSLPYTFGAGTKLELKRTVAAPSVFIFPPSDEQLKSGTASVVCLLNNFYPREAKVQWKVDNALQSGNSQESVTEQDSKDSTYSLSSTLTLSKADYEKHKVYACEVTHQGLSSPVTKSFNRGEC

SEQ ID NO: 9 - DNA, 690 bp, artificial
  VH of Fab6A10
caggtccagctgaaggagtccggtccaggtctggtccagcctagtgagaccctgtcactgacttgcaccgtgtcaggattctccctgaccacatacagtgtctcatgggtgagacagccttccgggaagggtccagaatggatggggaggatgtggtacgacggcgacacagtgtataacagcgccctgaaatctaggctgtccatcagccgggacacttctaagaaccaggtgtttctgaaaatgaattccctggagactgatgaaacaggcacttactattgcaccagggacttcgggtactttgatggttccagcccattcgactattggggccagggagtgatggtcaccgtgtctagtgctagtacaaaggggcccagcgtgtttccactggcaccctcatccaaatctactagtggaggaaccgccgctctgggctgtctggtgaaggattatttccccgagcctgtcaccgtgagctggaattctggcgcactgacaagcggagtccacacttttccagccgtgctgcagagctctggcctgtactccctgagttcagtggtcacagtcccctccagctctctgggaacccagacatacatctgtaacgtgaaccataagcctagcaacactaaggtggacaaaaaggtggagccaaaatcctgcgacaaaacccatacataa

SEQ ID NO: 10 - DNA, 657 bp, artificial
  VL of Fab6A10
agatgtcccgtcgatattgtgctgacccagagcccagccacactgagtgtgactcccggagagtctgtcagtctgtcatgcagggctagccaggggatctccaccagcattcactggtaccagcagaagagtaacgaatcacccaggctgctgatcaaattcgcctctcagagtatctcaggaattccatctcggttctccggcagcggatctgggactgactttaccctgtccattaatagagtggagagcgaagatttctctgtctatttttgccagcagacatacagcctgccctataccttcggtgcaggcacaaagctggagctgaaacgcactgtggccgctcctagcgtcttcatctttcccccttctgacgaacagctgaagagtggtacagcttcagtggtctgtctgctgaacaatttttacccacgagaggcaaaggtgcagtggaaagtcgataacgccctgcagtccggcaatagccaggagtctgtgactgaacaggacagtaaggattcaacctattccctgtccagcaccctgacactgtccaaagctgactacgagaagcataaagtgtatgcatgtgaagtcacccaccaggggctgtcatcacccgtcacaaaatcattcaataggggggagtgctaa

SEQ ID NO: 11 - protein, 248 aa, artificial
  VH of Fab6A10 with IgG secretion sequence
MYLGLNYVFIVFLLNGVQSQVQLKESGPGLVQPSETLSLTCTVSGFSLTTYSVSWVRQPSGKGPEWMGRMWYDGDTVYNSALKSRLSISRDTSKNQVFLKMNSLETDETGTYYCTRDFGYFDGSSPFDYWGQGVMVTVSSASTKGPSVFPLAPSSKSTSGGTAALGCLVKDYFPEPVTVSWNSGALTSGVHTFPAVLQSSGLYSLSSVVTVPSSSLGTQTYICNVNHKPSNTKVDKKVEPKSCDKTHT

SEQ ID NO: 12 - protein, 236 aa, artificial
  VL of Fab6A10 with IgL secretion sequence
MSVPTQVLGLLLLWLTDARCPVDIVLTQSPATLSVTPGESVSLSCRASQGISTSIHWYQQKSNESPRLLIKFASQSISGIPSRFSGSGSGTDFTLSINRVESEDFSVYFCQQTYSLPYTFGAGTKLELKRTVAAPSVFIFPPSDEQLKSGTASVVCLLNNFYPREAKVQWKVDNALQSGNSQESVTEQDSKDSTYSLSSTLTLSKADYEKHKVYACEVTHQGLSSPVTKSFNRGEC

SEQ ID NO: 13 - DNA, 747 bp, artificial
  VH of Fab6A10 with IgG secretion sequence
atgtatctgggtctgaactatgtctttatcgtctttctgctgaacggggtccagtcacaggtccagctgaaggagtccggtccaggtctggtccagcctagtgagaccctgtcactgacttgcaccgtgtcaggattctccctgaccacatacagtgtctcatgggtgagacagccttccgggaagggtccagaatggatggggaggatgtggtacgacggcgacacagtgtataacagcgccctgaaatctaggctgtccatcagccgggacacttctaagaaccaggtgtttctgaaaatgaattccctggagactgatgaaacaggcacttactattgcaccagggacttcgggtactttgatggttccagcccattcgactattggggccagggagtgatggtcaccgtgtctagtgctagtacaaaggggcccagcgtgtttccactggcaccctcatccaaatctactagtggaggaaccgccgctctgggctgtctggtgaaggattatttccccgagcctgtcaccgtgagctggaattctggcgcactgacaagcggagtccacacttttccagccgtgctgcagagctctggcctgtactccctgagttcagtggtcacagtcccctccagctctctgggaacccagacatacatctgtaacgtgaaccataagcctagcaacactaaggtggacaaaaaggtggagccaaaatcctgcgacaaaacccatacataa

SEQ ID NO: 14 - DNA, 711 bp, artificial
  VL of Fab6A10 with IgL secretion sequence
atgtccgtgcctacccaggtgctggggctgctgctgctgtggctgactgatgcaagatgtcccgtcgatattgtgctgacccagagcccagccacactgagtgtgactcccggagagtctgtcagtctgtcatgcagggctagccaggggatctccaccagcattcactggtaccagcagaagagtaacgaatcacccaggctgctgatcaaattcgcctctcagagtatctcaggaattccatctcggttctccggcagcggatctgggactgactttaccctgtccattaatagagtggagagcgaagatttctctgtctatttttgccagcagacatacagcctgccctataccttcggtgcaggcacaaagctggagctgaaacgcactgtggccgctcctagcgtcttcatctttcccccttctgacgaacagctgaagagtggtacagcttcagtggtctgtctgctgaacaatttttacccacgagaggcaaaggtgcagtggaaagtcgataacgccctgcagtccggcaatagccaggagtctgtgactgaacaggacagtaaggattcaacctattccctgtccagcaccctgacactgtccaaagctgactacgagaagcataaagtgtatgcatgtgaagtcacccaccaggggctgtcatcacccgtcacaaaatcattcaataggggggagtgctaa

SEQ ID NO: 15 - protein, 19 aa, artificial
  IgG secretion sequence
MYLGLNYVFIVFLLNGVQS

SEQ ID NO: 16 - protein, 20 aa, artificial
  IgL secretion sequence
MSVPTQVLGLLLLWLTDARC

SEQ ID NO: 17 - protein, 15 aa, artificial
  N-terminal fragment of the VL of Fab6A10
PVDIVLTQSPATLSV

SEQ ID NO: 18 - protein, 17 aa, artificial
  N-terminal fragment of the VL of Fab6A10
RCPVDIVLTQSPATLSV

SEQ ID NO: 19 - protein, 15 aa, artificial
  N-terminal fragment of the VH of Fab6A10
QVQLKESGPGLVQPS

SEQ ID NO: 20 - protein, 15 aa, artificial
  C-terminal fragment of the VL of Fab6A10
GLSSPVTKSFNRGEC

SEQ ID NO: 21 - protein, 15 aa, artificial
  C-terminal fragment of the VH of Fab6A10
VDKKVEPKSCDKTHT